European Patent Specification EP 3 445 876 B1, published July 5, 2023. Title: SINGLE CELL ANALYSIS OF TRANSPOSASE ACCESSIBLE CHROMATIN. Applicant: 10X GENOMICS, INC. Application Regional processing of PCT/US18/34774. The sequence listing filed with the application follows.

SEQUENCE LISTING (20 sequences)

SEQ ID NO: 1 - DNA, 18 bp, Artificial Sequence
  Description of Artificial Sequence: Synthetic oligonucleotide
agatgtgtataagagaca

SEQ ID NO: 2 - DNA, 36 bp, Artificial Sequence
  Description of Artificial Sequence: Synthetic oligonucleotide
tctacactctttccctacacgacgctcttccgatct

SEQ ID NO: 3 - DNA, 33 bp, Artificial Sequence
  Description of Artificial Sequence: Synthetic oligonucleotide
tcgtcggcagcgtcagatgtgtataagagacag

SEQ ID NO: 4 - DNA, 23 bp, Artificial Sequence
  Description of Artificial Sequence: Synthetic oligonucleotide
actacacgacgctcttccgatct

SEQ ID NO: 5 - DNA, 34 bp, Artificial Sequence
  Description of Artificial Sequence: Synthetic oligonucleotide
gtgactggagttcagacgtgtgctcttccgatct

SEQ ID NO: 6 - DNA, 34 bp, Artificial Sequence
  Description of Artificial Sequence: Synthetic oligonucleotide
gtctcgtgggctcggagatgtgtataagagacag

SEQ ID NO: 7 - DNA, 18 bp, Artificial Sequence
  Description of Artificial Sequence: Synthetic oligonucleotide
taatacgactcactatag

SEQ ID NO: 8 - DNA, 67 bp, Artificial Sequence
  Description of Artificial Sequence: Synthetic oligonucleotide
  modified_base (37)..(48): a, c, t, g, unknown or other
tctacactctttccctacacgacgctcttccgatctnnnnnnnnnnnnagatgtgtataagagacag

SEQ ID NO: 9 - DNA, 65 bp, Artificial Sequence
  Description of Artificial Sequence: Synthetic oligonucleotide
  modified_base (20)..(31): a, c, t, g, unknown or other
ctgtctcttatacacatctnnnnnnnnnnnnagatcggaagagcacacgtctgaactccagtcac

SEQ ID NO: 10 - DNA, 87 bp, Artificial Sequence
  Description of Artificial Sequence: Synthetic oligonucleotide
  modified_base (57)..(68): a, c, t, g, unknown or other
aatgatacggcgaccaccgatctacactctttccctacacgacgctcttccgatctnnnnnnnnnnnnagatgtgtataagagacag

SEQ ID NO: 11 - DNA, 97 bp, Artificial Sequence
  Description of Artificial Sequence: Synthetic oligonucleotide
  modified_base (20)..(31): a, c, t, g, unknown or other
  modified_base (66)..(73): a, c, t, g, unknown or other
ctgtctcttatacacatctnnnnnnnnnnnnagatcggaagagcacacgtctgaactccagtcacnnnnnnnnatctcgtatgccgtcttctgcttg

SEQ ID NO: 12 - DNA, 48 bp, Artificial Sequence
  Description of Artificial Sequence: Synthetic oligonucleotide
  modified_base (37)..(48): a, c, t, g, unknown or other
tctacactctttccctacacgacgctcttccgatctnnnnnnnnnnnn

SEQ ID NO: 13 - DNA, 46 bp, Artificial Sequence
  Description of Artificial Sequence: Synthetic oligonucleotide
  modified_base (1)..(12): a, c, t, g, unknown or other
nnnnnnnnnnnnagatcggaagagcacacgtctgaactccagtcac

SEQ ID NO: 14 - DNA, 19 bp, Artificial Sequence
  Description of Artificial Sequence: Synthetic oligonucleotide
agatgtgtataagagacag

SEQ ID NO: 15 - DNA, 19 bp, Artificial Sequence
  Description of Artificial Sequence: Synthetic oligonucleotide
ctgtctcttatacacatct

SEQ ID NO: 16 - DNA, 68 bp, Artificial Sequence
  Description of Artificial Sequence: Synthetic oligonucleotide
  modified_base (57)..(68): a, c, t, g, unknown or other
aatgatacggcgaccaccgatctacactctttccctacacgacgctcttccgatctnnnnnnnnnnnn

SEQ ID NO: 17 - DNA, 78 bp, Artificial Sequence
  Description of Artificial Sequence: Synthetic oligonucleotide
  modified_base (1)..(12): a, c, t, g, unknown or other
  modified_base (47)..(54): a, c, t, g, unknown or other
nnnnnnnnnnnnagatcggaagagcacacgtctgaactccagtcacnnnnnnnnatctcgtatgccgtcttctgcttg

SEQ ID NO: 18 - DNA, 97 bp, Artificial Sequence; identical to SEQ ID NO: 11
  Description of Artificial Sequence: Synthetic oligonucleotide
  modified_base (20)..(31): a, c, t, g, unknown or other
  modified_base (66)..(73): a, c, t, g, unknown or other

SEQ ID NO: 19 - DNA, 87 bp, Artificial Sequence
  Description of Artificial Sequence: Synthetic oligonucleotide
  modified_base (53)..(68): a, c, t, g, unknown or other
cgatgacgttaatacgactcactatagggactacacgacgctcttccgatctnnnnnnnnnnnnnnnnagatgtgtataagagacag

SEQ ID NO: 20 - DNA, 53 bp, Artificial Sequence
  Description of Artificial Sequence: Synthetic oligonucleotide
  modified_base (23)..(34): a, c, t, g, unknown or other
ctacacgacgctcttccgatctnnnnnnnnnnnnagatgtgtataagagacag